European Patent Application EP 4 635 973 A1, published October 22, 2025. Title: synthetic peptide and construct. Applicant: TOAGOSEI CO., LTD. The sequence listing filed with the application follows.

SEQUENCE LISTING (11 sequences)

SEQ ID NO: 1 - protein, 4 aa, synthetic construct
PDPD

SEQ ID NO: 2 - protein, 4 aa, synthetic construct
PEPE

SEQ ID NO: 3 - protein, 4 aa, synthetic construct
PDPE

SEQ ID NO: 4 - protein, 4 aa, synthetic construct
PEPD

SEQ ID NO: 5 - protein, 5 aa, synthetic construct
PDPDG

SEQ ID NO: 6 - protein, 5 aa, synthetic construct
PEPEG

SEQ ID NO: 7 - protein, 5 aa, synthetic construct
PDPEG

SEQ ID NO: 8 - protein, 5 aa, synthetic construct
PEPDG

SEQ ID NO: 9 - protein, 13 aa, synthetic construct
PDPDPDPDPDPDG

SEQ ID NO: 10 - protein, 13 aa, synthetic construct
PEPEPEPEPEPEG

SEQ ID NO: 11 - protein, 13 aa, synthetic construct
PDPEPDPEPDPEG